European Patent Specification EP 3 774 858 B1, published July 30, 2025. Title: C-terminal CDNF and MANF fragments, pharmaceutical compositions comprising same and uses thereof. Applicant: Helsingin yliopisto. The sequence listing filed with the application follows.

SEQUENCE LISTING (24 sequences)

SEQ ID NO: 1 - protein, 81 aa, Homo sapiens [sequence omitted]

SEQ ID NO: 2 - protein, 78 aa, Homo sapiens
ICEKLKKKDSQICELKYDKQIDLSTVDLKKLRVKELKKILDDWGETCKGCAEKSDYIRKINELMPKYAPKAASARTDL

SEQ ID NO: 3 - protein, 81 aa, Homo sapiens
  misc_feature (53)..(54): Xaa can be any naturally occurring amino acid
MPAMKICEKLKKLDSQICELKYEKTLDLASVDLRKMRVAELKQILHSWGEECXXCAEKTDYVNLIQELAPKYAATHPKTEL

SEQ ID NO: 4 - protein, 61 aa, Homo sapiens
KYEKTLDLASVDLRKMRVAELKQILHSWGEECRACAEKTDYVNLIQELAPKYAATHPKTEL

SEQ ID NO: 5 - protein, 63 aa, Homo sapiens
KYDKQIDLSTVDLKKLRVKELKKILDDWGETCKGCAEKSDYIRKINELMPKYAPKAASARTDL

SEQ ID NO: 6 - protein, 68 aa, Homo sapiens
  misc_feature (38)..(39): Xaa can be any naturally occurring amino acid
QICELKYDKQIDLSTVDLKKLRVKELKKILDDWGETCXXCAEKSDYIRKINELMPKYAPKAASARTDL

SEQ ID NO: 7 - protein, 161 aa, Homno sapiens
QEAGGRPGADCEVCKEFLNRFYKSLIDRGVNFSLDTIEKELISFCLDTKGKENRLCYYLGATKDAATKILSEVTRPMSVHMPAMKICEKLKKLDSQICELKYEKTLDLASVDLRKMRVAELKQILHSWGEECRACAEKTDYVNLIQELAPKYAATHPKTEL

SEQ ID NO: 8 - protein, 100 aa, Homo sapiens
QEAGGRPGADCEVCKEFLNRFYKSLIDRGVNFSLDTIEKELISFCLDTKGKENRLCYYLGATKDAATKILSEVTRPMSVHMPAMKICEKLKKLDSQICEL

SEQ ID NO: 9 - protein, 158 aa, Homo sapiens
LRPGDCEVCISYLGRFYQDLKDRDVTFSPATIENELIKFCREARGKENRLCYYIGATDDAATKIINEVSKPLAHHIPVEKICEKLKKKDSQICELKYDKQIDLSTVDLKKLRVKELKKILDDWGETCKGCAEKSDYIRKINELMPKYAPKAASARTDL

SEQ ID NO: 10 - protein, 95 aa, Homo sapiens
LRPGDCEVCISYLGRFYQDLKDRDVTFSPATIENELIKFCREARGKENRLCYYIGATDDAATKIINEVSKPLAHHIPVEKICEKLKKKDSQICEL

SEQ ID NO: 11 - protein, 57 aa, Homo sapiens
TLDLASVDLRKMRVAELKQILHSWGEECRACAEKTDYVNLIQELAPKYAATHPKTEL

SEQ ID NO: 12 - protein, 53 aa, Homo sapiens
KYEKTLDLASVDLRKMRVAELKQILHSWGEECRACAEKTDYVNLIQELAPKYA

SEQ ID NO: 13 - protein, 49 aa, Homo sapiens
TLDLASVDLRKMRVAELKQILHSWGEECRACAEKTDYVNLIQELAPKYA

SEQ ID NO: 14 - protein, 51 aa, Homo sapiens
VDLRKMRVAELKQILHSWGEECRACAEKTDYVNLIQELAPKYAATHPKTEL

SEQ ID NO: 15 - protein, 43 aa, Homo sapiens
VDLRKMRVAELKQILHSWGEECRACAEKTDYVNLIQELAPKYA

SEQ ID NO: 16 - protein, 50 aa, Homo sapiens
KYEKTLDLASVDLRKMRVAELKQILHSWGEECRACAEKTDYVNLIQELAP

SEQ ID NO: 17 - protein, 37 aa, Homo sapiens
RVAELKQILHSWGEECRACAEKTDYVNLIQELAPKYA

SEQ ID NO: 18 - protein, 49 aa, Artificial
  C-CDNF peptide with single amino acid substitution
TLDLASVDLRKMRVAELKQILHSWGEESRACAEKTDYVNLIQELAPKYA

SEQ ID NO: 19 - protein, 49 aa, Artificial
  C-CDNF peptide with single amino acid substitution
TLDLASVDLRKMRVAELKQILHSWGEECRASAEKTDYVNLIQELAPKYA

SEQ ID NO: 20 - protein, 51 aa, Artificial
  Mutated C-CDNF peptide
TLDLASVDLRKMRVAELKQILHSWGEECRARACAEKTDYVNLIQELAPKYA

SEQ ID NO: 21 - protein, 49 aa, Artificial
  Mutated C-CDNF peptide
TLDLASVDLRKMRVAEPKQILHSWGEECRACAEKTDYVNLIQELAPKYA

SEQ ID NO: 22 - protein, 49 aa, Artificial
  Mutated C-CDNF peptide
TLDLASVDLRKMRVAELKQILHSWGEECRACAEKTDYVNLIQEPAPKYA

SEQ ID NO: 23 - protein, 49 aa, Artificial
  Mutated C-CDNF peptide
TLDLASVDLRKMRVAEPKQILHSWGEECRACAEKTDYVNLIQEPAPKYA

SEQ ID NO: 24 - protein, 33 aa, Homo sapiens
TLDLASVDLRKMRVAELKQILHSWGEECRACAE